European Patent Application EP 4 803 097 A1, published September 9, 2026. Title: 一种用于预防结核分枝杆菌感染的纳米颗粒疫苗及其制备方法. Applicant: 烟台派诺生物技术有限公司. The sequence listing filed with the application follows.

SEQUENCE LISTING (31 sequences)

SEQ ID NO: 1 - protein, 13 aa, synthetic construct
AHIVMVDAYKPTK

SEQ ID NO: 2 - protein, 6 aa, synthetic construct
GSGGSG

SEQ ID NO: 3 - protein, 324 aa, synthetic construct
MAPPALSQDRFADFPALPLDPSAMVAQVGPQVVNINTKLGYNNAVGAGTGIVIDPNGVVLTNNHVIAGATDINAFSVGSGQTYGVDVVGYDRTQDVAVLQLRGAGGLPSAAIGGGVAVGEPVVAMGNSGGQGGTPRAVPGRVVALGQTVQASDSLTGAEETLNGLIQFDAAIQPGDAGGPVVNGLGQVVGMNTAASDNFQLSQGGQGFAIPIGQAMAIAGQIRSGGGSPTVHIGPTAFLGLGVVDNNGNGARVQRVVGSAPAASLGISTGDVITAVDGAPINSATAMADALNGHHPGDVISVTWQTKSGGTRTGNVTLAEGPPA

SEQ ID NO: 4 - protein, 349 aa, synthetic construct
MAPPALSQDRFADFPALPLDPSAMVAQVGPQVVNINTKLGYNNAVGAGTGIVIDPNGVVLTNNHVIAGATDINAFSVGSGQTYGVDVVGYDRTQDVAVLQLRGAGGLPSAAIGGGVAVGEPVVAMGNSGGQGGTPRAVPGRVVALGQTVQASDSLTGAEETLNGLIQFDAAIQPGDAGGPVVNGLGQVVGMNTAASDNFQLSQGGQGFAIPIGQAMAIAGQIRSGGGSPTVHIGPTAFLGLGVVDNNGNGARVQRVVGSAPAASLGISTGDVITAVDGAPINSATAMADALNGHHPGDVISVTWQTKSGGTRTGNVTLAEGPPAGSGGSGAHIVMVDAYKPTKHHHHHH

SEQ ID NO: 5 - protein, 297 aa, synthetic construct
MAFSRPGLPVEYLQVPSPSMGRDIKVQFQSGGANSPALYLLDGLRAQDDFSGWDINTPAFEWYDQSGLSVVMPVGGQSSFYSDWYQPACGKAGCQTYKWETFLTSELPGWLQANRHVKPTGSAVVGLSMAASSALTLAIYHPQQFVYAGAMSGLLDPSQAMGPTLIGLAMGDAGGYKASDMWGPKEDPAWQRNDPLLNVGKLIANNTRVWVYCGNGKPSDLGGNNLPAKFLEGFVRTSNIKFQDAYNAGGGHNGVFDFPDSGTHSWEYWGAQLNAMKPDLQRALGATPNTGPAPQGA

SEQ ID NO: 6 - protein, 322 aa, synthetic construct
MAFSRPGLPVEYLQVPSPSMGRDIKVQFQSGGANSPALYLLDGLRAQDDFSGWDINTPAFEWYDQSGLSVVMPVGGQSSFYSDWYQPACGKAGCQTYKWETFLTSELPGWLQANRHVKPTGSAVVGLSMAASSALTLAIYHPQQFVYAGAMSGLLDPSQAMGPTLIGLAMGDAGGYKASDMWGPKEDPAWQRNDPLLNVGKLIANNTRVWVYCGNGKPSDLGGNNLPAKFLEGFVRTSNIKFQDAYNAGGGHNGVFDFPDSGTHSWEYWGAQLNAMKPDLQRALGATPNTGPAPQGAGSGGSGAHIVMVDAYKPTKHHHHHH

SEQ ID NO: 7 - protein, 200 aa, synthetic construct
MTEQQWNFAGIEAAASAIQGNVTSIHSLLDEGKQSLTKLAAAWGGSGSEAYQGVQQKWDATATELNNALQNLARTISEAGQAMASTEGNVTGMFAGSGGSGAEMKTDAATLAQEAGNFERISGDLKTQIDQVESTAGSLQGQWRGAAGTAAQAAVVRFQEAANKQKQELDEISTNIRQAGVQYSRADEEQQQALSSQMGF

SEQ ID NO: 8 - protein, 225 aa, synthetic construct
MTEQQWNFAGIEAAASAIQGNVTSIHSLLDEGKQSLTKLAAAWGGSGSEAYQGVQQKWDATATELNNALQNLARTISEAGQAMASTEGNVTGMFAGSGGSGAEMKTDAATLAQEAGNFERISGDLKTQIDQVESTAGSLQGQWRGAAGTAAQAAVVRFQEAANKQKQELDEISTNIRQAGVQYSRADEEQQQALSSQMGFGSGGSGAHIVMVDAYKPTKHHHHHH

SEQ ID NO: 9 - protein, 176 aa, synthetic construct
MIAGVDQALAATGQASQRAAGASGGVTVGVGVGTEQRNLSVVAPSQFTFSSRSPDFVDETAGQSWAAILGLNQFHGSGGSGSQIMYNYPAMLGHAGDMAGYAGTLQSLGAEIAVEQAALQSAWQGDTGITYQAWQAQWNQAMEDLVRAYHAMSSTHEANTMAMMARDTAEAAKWGG

SEQ ID NO: 10 - protein, 201 aa, synthetic construct
MIAGVDQALAATGQASQRAAGASGGVTVGVGVGTEQRNLSVVAPSQFTFSSRSPDFVDETAGQSWAAILGLNQFHGSGGSGSQIMYNYPAMLGHAGDMAGYAGTLQSLGAEIAVEQAALQSAWQGDTGITYQAWQAQWNQAMEDLVRAYHAMSSTHEANTMAMMARDTAEAAKWGGGSGGSGAHIVMVDAYKPTKHHHHHH

SEQ ID NO: 11 - protein, 748 aa, synthetic construct
MHHHHHHAHIVMVDAYKPTKGSGGSGTAASDNFQLSQGGQGFAIPIGQAMAIAGQIRSGGGSPTVHIGPTAFLGLGVVDNNGNGARVQRVVGSAPAASLGISTGDVITAVDGAPINSATAMADALNGHHPGDVISVTWQTKSGGTRTGNVTLAEGPPAEFMVDFGALPPEINSARMYAGPGSASLVAAAQMWDSVASDLFSAASAFQSVVWGLTVGSWIGSSAGLMVAAASPYVAWMSVTAGQAELTAAQVRVAAAAYETAYGLTVPPPVIAENRAELMILIATNLLGQNTPAIAVNEAEYGEMWAQDAAAMFGYAAATATATATLLPFEEAPEMTSAGGLLEQAAAVEEASDTAAANQLMNNVPQALQQLAQPTQGTTPSSKLGGLWKTVSPHRSPISNMVSMANNHMSMTNSGVSMTNTLSSMLKGFAPAAAAQAVQTAAQNGVRAMSSLGSSLGSSGLGGGVAANLGRAASVGSLSVPQAWAAANQAVTPAARALPLTSLTSAAERGPGQMLGGLPVGQMGARAGGGLSGVLRVPPRPYVMPHSPAAGDIAPPALSQDRFADFPALPLDPSAMVAQVGPQVVNINTKLGYNNAVGAGTGIVIDPNGVVLTNNHVIAGATDINAFSVGSGQTYGVDVVGYDRTQDVAVLQLRGAGGLPSAAIGGGVAVGEPVVAMGNSGGQGGTPRAVPGRVVALGQTVQASDSLTGAEETLNGLIQFDAAIQPGDAGGPVVNGLGQVVGMNTAAS

SEQ ID NO: 12 - DNA, 39 bp, synthetic construct
  source 1..39: mol_type = other DNA
gcccacattgttatggtggacgcatacaaaccgaccaaa

SEQ ID NO: 13 - DNA, 18 bp, synthetic construct
  source 1..18: mol_type = other DNA
ggttccggcggttctggt

SEQ ID NO: 14 - DNA, 18 bp, synthetic construct
  source 1..18: mol_type = other DNA
caccaccaccatcaccac

SEQ ID NO: 15 - DNA, 972 bp, synthetic construct
  source 1..972: mol_type = other DNA
atggctccgcctgcactgtcccaggaccgtttcgctgacttccctgctctgccgctggatccgtctgcgatggtggctcaggtcggcccgcaggtggtcaacattaacaccaaactgggctataacaacgctgttggtgcgggtactggtatcgtgatcgatccgaacggtgttgtgctgactaacaaccacgtgatcgctggcgctacggacatcaacgccttctccgtcggtagcggtcaaacctatggtgtcgacgtggtcggctacgatcgtacccaggacgttgctgttctgcagctgcgtggtgctggcggcctgccgtctgccgctattggtggtggtgtggcagtaggtgagccagtggtggctatgggcaactctggtggccagggtggcactcctcgtgcggtaccaggccgtgtcgtggctctgggccagactgttcaggccagcgacagcctgactggcgcggaagagactctgaatggcctgatccagttcgacgctgcaatccaaccgggcgatgcgggcggtcctgtagtaaacggcctgggtcaggtagtgggtatgaacaccgctgctagcgataatttccaactgagccagggcggccagggtttcgcaatccctattggccaggccatggcaatcgcaggccagatccgtagcggtggtggctccccgacggtacatatcggtccgaccgcgttcctgggcctgggcgtggtggacaataacggcaacggtgcgcgtgtgcaacgtgtagtcggctccgctccagcagcttccctgggtatcagcactggtgacgtcattactgctgtcgatggtgcgccgatcaactctgctactgcgatggcagatgcactgaacggtcaccaccctggcgacgttatctccgttacgtggcagacgaaatccggtggcacccgtacgggcaacgtgaccctggcggaaggcccgccggca

SEQ ID NO: 16 - DNA, 1045 bp, synthetic construct
  source 1..1045: mol_type = other DNA
atggctccgcctgcactgtcccaggaccgtttcgctgacttccctgctctgccgctggatccgtctgcgatggtggctcaggtcggcccgcaggtggtcaacattaacaccaaactgggctataacaacgctgttggtgcgggtactggtatcgtgatcgatccgaacggtgttgtgctgactaacaaccacgtgatcgctggcgctacggacatcaacgccttctccgtcggtagcggtcaaacctatggtgtcgacgtggtcggctacgatcgtacccaggacgttgctgttctgcagctgcgtggtgctggcggcctgccgtctgccgctattggtggtggtgtggcagtaggtgagccagtggtggctatgggcaactctggtggccagggtggcactcctcgtgcggtaccaggccgtgtcgtggctctgggccagactgttcaggccagcgacagcctgactggcgcggaagagactctgaatggcctgatccagttcgacgctgcaatccaaccgggcgatgcgggcggtcctgtagtaaacggcctgggtcaggtagtgggtatgaacaccgctgctagcgataatttccaactgagccagggcggccagggtttcgcaatccctattggccaggccatggcaatcgcaggccagatccgtagcggtggtggctccccgacggtacatatcggtccgaccgcgttcctgggcctgggcgtggtggacaataacggcaacggtgcgcgtgtgcaacgtgtagtcggctccgctccagcagcttccctgggtatcagcactggtgacgtcattactgctgtcgatggtgcgccgatcaactctgctactgcgatggcagatgcactgaacggtcaccaccctggcgacgttatctccgttacgtggcagacgaaatccggtggcacccgtacgggcaacgtgaccctggcggaaggcccgccggcaggttccggcggttctggtgcccacattgttatggtggacgcatacaaaccgaccaaacaccaaccatcaccac

SEQ ID NO: 17 - DNA, 891 bp, synthetic construct
  source 1..891: mol_type = other DNA
atggccttctcccgccctggtctgccggtcgaatatctgcaagttccgagcccgtctatgggtcgcgacattaaagttcagttccagtccggcggcgcaaactcccctgcgctgtatctgctggatggtctgcgcgcacaggacgacttttccggctgggatatcaacaccccggcattcgagtggtatgaccagtccggtctgtccgttgttatgccggttggcggtcagtcctccttctattctgactggtaccagccggcctgcggcaaagctggttgccagacgtacaaatgggaaaccttcctgacgtccgaactgccaggctggctgcaggcgaaccgtcacgtcaagccgaccggttctgcagtagtaggtctgtctatggctgcctcctctgctctgactctggctatctaccacccgcagcaattcgtgtacgcgggtgcgatgagcggtctgctggacccgagccaagctatgggtccaaccctgatcggtctggcaatgggcgatgcgggtggctataaagcttccgacatgtggggcccaaaagaagatccagcctggcaacgtaacgacccgctgctgaacgtcggcaaactgatcgctaacaacacccgcgtatgggtatactgtggtaacggtaagccgagcgacctgggtggtaacaacctgccggcgaaattcctggaaggttttgtgcgtacgagcaacatcaagttccaagacgcgtataacgctggcggcggtcacaacggtgtcttcgatttcccggactccggcacccattcctgggaatattggggcgcccagctgaacgctatgaaacctgatctgcaacgtgccctgggcgcaacgccaaacaccggtccagctccgcagggtgct

SEQ ID NO: 18 - DNA, 966 bp, synthetic construct
  source 1..966: mol_type = other DNA
atggccttctcccgccctggtctgccggtcgaatatctgcaagttccgagcccgtctatgggtcgcgacattaaagttcagttccagtccggcggcgcaaactcccctgcgctgtatctgctggatggtctgcgcgcacaggacgacttttccggctgggatatcaacaccccggcattcgagtggtatgaccagtccggtctgtccgttgttatgccggttggcggtcagtcctccttctattctgactggtaccagccggcctgcggcaaagctggttgccagacgtacaaatgggaaaccttcctgacgtccgaactgccaggctggctgcaggcgaaccgtcacgtcaagccgaccggttctgcagtagtaggtctgtctatggctgcctcctctgctctgactctggctatctaccacccgcagcaattcgtgtacgcgggtgcgatgagcggtctgctggacccgagccaagctatgggtccaaccctgatcggtctggcaatgggcgatgcgggtggctataaagcttccgacatgtggggcccaaaagaagatccagcctggcaacgtaacgacccgctgctgaacgtcggcaaactgatcgctaacaacacccgcgtatgggtatactgtggtaacggtaagccgagcgacctgggtggtaacaacctgccggcgaaattcctggaaggttttgtgcgtacgagcaacatcaagttccaagacgcgtataacgctggcggcggtcacaacggtgtcttcgatttcccggactccggcacccattcctgggaatattggggcgcccagctgaacgctatgaaacctgatctgcaacgtgccctgggcgcaacgccaaacaccggtccagctccgcagggtgctggttccggcggttctggtgcccacattgttatggtggacgcatacaaaccgaccaaacaccaccaccatcaccac

SEQ ID NO: 19 - DNA, 600 bp, synthetic construct
  source 1..600: mol_type = other DNA
atgaccgaacagcagtggaacttcgcgggcattgaagcagcagcatctgcaatccagggcaacgttacttccattcactctctgctggacgagggtaagcagtctctgaccaaactggcagcggcgtggggcggttctggttctgaggcttaccagggcgtgcagcagaaatgggacgcgactgcgactgagctgaacaacgctctgcagaacctggctcgtactatcagcgaggccggtcaagcgatggcgtctacggaaggtaacgtgaccggcatgttcgcgggttccggtggtagcggtgcggagatgaaaaccgatgccgcgactctggcacaggaagctggtaacttcgaacgcattagcggtgacctgaagacccagatcgatcaggtcgaatccaccgccggcagcctgcaaggtcagtggcgtggcgctgcaggcacggcggcccaagcagctgtggttcgtttccaggaagctgcgaacaaacagaaacaggagctggacgagatctctacgaacatccgtcaggctggtgtgcagtattcccgtgcagacgaagaacagcaacaggcgctgtctagccagatgggcttt

SEQ ID NO: 20 - DNA, 675 bp, synthetic construct
  source 1..675: mol_type = other DNA
atgaccgaacagcagtggaacttcgcgggcattgaagcagcagcatctgcaatccagggcaacgttacttccattcactctctgctggacgagggtaagcagtctctgaccaaactggcagcggcgtggggcggttctggttctgaggcttaccagggcgtgcagcagaaatgggacgcgactgcgactgagctgaacaacgctctgcagaacctggctcgtactatcagcgaggccggtcaagcgatggcgtctacggaaggtaacgtgaccggcatgttcgcgggttccggtggtagcggtgcggagatgaaaaccgatgccgcgactctggcacaggaagctggtaacttcgaacgcattagcggtgacctgaagacccagatcgatcaggtcgaatccaccgccggcagcctgcaaggtcagtggcgtggcgctgcaggcacggcggcccaagcagctgtggttcgtttccaggaagctgcgaacaaacagaaacaggagctggacgagatctctacgaacatccgtcaggctggtgtgcagtattcccgtgcagacgaagaacagcaacaggcgctgtctagccagatgggctttggttccggcggttctggtgcccacattgttatggtggacgcatacaaaccgaccaaacaccaccaccatcaccac

SEQ ID NO: 21 - DNA, 528 bp, synthetic construct
  source 1..528: mol_type = other DNA
atgattgcaggcgtggatcaggcactggcagcgaccggtcaggcatctcagcgtgcggccggcgccagcggcggtgttacggttggcgttggcgtgggtaccgaacagcgcaacctgtccgtggtggctccgtctcaattcacgttcagctcccgctccccggattttgtcgacgaaactgcgggtcagagctgggctgctatcctgggcctgaaccagtttcacggctccggtggcagcggctcccagatcatgtacaactacccggccatgctgggtcatgcgggtgatatggcaggctacgcaggtactctgcagtctctgggcgcggaaatcgcggttgaacaggctgcactgcagtctgcatggcagggtgacaccggcatcacgtatcaggcttggcaggcgcagtggaatcaggccatggaagacctggtacgtgcgtaccacgcgatgtcctctacgcatgaagcgaacaccatggccatgatggctcgtgacaccgcagaagcagcgaaatggggcggc

SEQ ID NO: 22 - DNA, 603 bp, synthetic construct
  source 1..603: mol_type = other DNA
atgattgcaggcgtggatcaggcactggcagcgaccggtcaggcatctcagcgtgcggccggcgccagcggcggtgttacggttggcgttggcgtgggtaccgaacagcgcaacctgtccgtggtggctccgtctcaattcacgttcagctcccgctccccggattttgtcgacgaaactgcgggtcagagctgggctgctatcctgggcctgaaccagtttcacggctccggtggcagcggctcccagatcatgtacaactacccggccatgctgggtcatgcgggtgatatggcaggctacgcaggtactctgcagtctctgggcgcggaaatcgcggttgaacaggctgcactgcagtctgcatggcagggtgacaccggcatcacgtatcaggcttggcaggcgcagtggaatcaggccatggaagacctggtacgtgcgtaccacgcgatgtcctctacgcatgaagcgaacaccatggccatgatggctcgtgacaccgcagaagcagcgaaatggggcggcggttccggcggttctggtgcccacattgttatggtggacgcatacaaaccgaccaaacaccaccaccatcaccac

SEQ ID NO: 23 - DNA, 2244 bp, synthetic construct
  source 1..2244: mol_type = other DNA
atgcaccaccaccatcaccacgcccacattgttatggtggacgcatacaaaccgaccaaaggttccggcggttctggtactgccgcgtccgataactttcagctgtcccaaggtggtcaaggtttcgcgattccgattggccaagcgatggctatcgcaggccaaatccgttccggtggcggttccccgactgtccacatcggtccgaccgctttcctgggcctgggcgtggttgacaacaatggtaacggtgcacgcgttcagcgcgttgttggctccgcgcctgcagcgagcctgggcatcagcaccggcgatgtaattaccgcagttgatggcgcgccgatcaattctgccaccgctatggctgacgcgctgaacggtcaccacccgggcgacgtcatctccgttacttggcagactaaaagcggtggtacccgtaccggcaacgttaccctggcggaaggtccaccggcggaattcatggttgacttcggtgcactgccgccggaaatcaatagcgcccgcatgtacgcaggtccgggttccgcgtctctggttgcggcagcccagatgtgggactctgttgcgagcgacctgttctccgcggcctccgcattccagtccgtagtttggggtctgacggttggttcctggatcggttcctctgcgggcctgatggtcgctgctgcgagcccgtacgttgcgtggatgtccgttaccgctggtcaggccgaactgaccgcggctcaggtccgtgtagcggcggcggcatacgagaccgcctacggcctgactgtgccgccacctgtcatcgcagagaatcgtgcggagctgatgattctgatcgcgacgaacctgctgggtcagaatactccggctatcgctgtcaacgaggcggaatacggcgaaatgtgggctcaggacgcagccgcaatgtttggttatgctgctgcaaccgcgaccgccaccgctaccctgctgccgttcgaagaggccccggaaatgacgtctgcaggtggtctgctggaacaagctgctgccgtggaggaggcgtctgacaccgcggctgctaatcagctgatgaacaacgtgccgcaggcactgcagcagctggcgcagccgactcaaggcacgaccccgtcttctaagctgggcggtctgtggaaaaccgtatccccgcatcgtagcccgattagcaacatggttagcatggcgaacaaccatatgtccatgactaactccggcgtgagcatgaccaacaccctgtcctctatgctgaaaggtttcgccccggcggctgccgcccaagctgtccagaccgcagctcagaacggcgttcgtgcgatgtcctccctgggctcttccctgggctcttctggcctgggtggtggcgttgctgctaatctgggccgcgcagcaagcgtcggtagcctgtctgtcccgcaggcatgggcagccgcgaaccaggctgtgactcctgccgcacgcgctctgccgctgacttccctgacgtctgccgcagaacgtggtccgggccagatgctgggtggtctgccagtaggtcagatgggtgcccgtgcgggtggtggtctgtccggtgttctgcgtgtaccaccgcgtccgtacgtcatgccgcactccccggccgcgggtgacatcgccccaccggcgctgagccaagaccgcttcgcggactttcctgctctgccgctggacccgtccgctatggttgcacaagtgggtccgcaggtggtgaacatcaacaccaaactgggttacaacaacgctgttggtgctggtactggtatcgtaatcgacccgaacggcgtggtactgaccaacaaccacgttatcgccggtgccaccgatatcaacgctttctctgtaggcagcggtcagacctacggcgtggatgttgttggctacgatcgcacccaggacgttgccgttctgcagctgcgcggtgctggtggtctgccgtctgctgccatcggcggcggcgttgccgtgggcgaaccggtagtagcaatgggcaactccggcggtcagggtggcactcctcgtgccgtgccgggccgcgtagtagctctgggtcagacggttcaggctagcgattctctgaccggcgcagaagaaaccctgaacggcctgattcagttcgacgctgcgattcaaccgggtgatgcgggcggtccggtagtgaacggcctgggccaggtggtgggcatgaacaccgctgcaagc

SEQ ID NO: 24 - protein, 93 aa, synthetic construct
MDSATHIKFSKRDEDGKELAGATMELRDSSGKTISTWISDGQVKDFYLYPGKYTFVETAAPDGYEVATAITFTVNEQGQVTVNGKATKGDAHI

SEQ ID NO: 25 - protein, 12 aa, synthetic construct
GGSGGSGGSGGS

SEQ ID NO: 26 - protein, 205 aa, synthetic construct
MKMEELFKKHKIVAVLRANSVEEAKKKALAVFLGGVHLIEITFTVPDADTVIKELSFLKEMGAIIGAGTVTSVEQARKAVESGAEFIVSPHLDEEISQFAKEKGVFYMPGVMTPTELVKAMKLGHTILKLFPGEVVGPQFVKAMKGPFPNVKFVPTGGVNLDNVCEWFKAGVLAVGVGSALVKGTPVEVAEKAKAFVEKIRGCTE

SEQ ID NO: 27 - protein, 310 aa, synthetic construct
MDSATHIKFSKRDEDGKELAGATMELRDSSGKTISTWISDGQVKDFYLYPGKYTFVETAAPDGYEVATAITFTVNEQGQVTVNGKATKGDAHIGGSGGSGGSGGSMKMEELFKKHKIVAVLRANSVEEAKKKALAVFLGGVHLIEITFTVPDADTVIKELSFLKEMGAIIGAGTVTSVEQARKAVESGAEFIVSPHLDEEISQFAKEKGVFYMPGVMTPTELVKAMKLGHTILKLFPGEVVGPQFVKAMKGPFPNVKFVPTGGVNLDNVCEWFKAGVLAVGVGSALVKGTPVEVAEKAKAFVEKIRGCTE

SEQ ID NO: 28 - DNA, 279 bp, synthetic construct
  source 1..279: mol_type = other DNA
atggactctgctactcacatcaaattctctaaacgcgacgaagacggcaaagaactggcaggcgctactatggaactgcgtgactccagcggcaaaactatctccacttggatctccgacggtcaggtgaaggatttctacctgtacccgggcaaatacaccttcgttgaaactgcagcacctgacggttacgaagtagcaactgctatcacgttcaccgttaacgagcagggtcaggttaccgttaacggcaaggcgactaagggtgatgcacacatc

SEQ ID NO: 29 - DNA, 36 bp, synthetic construct
  source 1..36: mol_type = other DNA
ggtggttctggcggctctggtggttctggtggctct

SEQ ID NO: 30 - DNA, 615 bp, synthetic construct
  source 1..615: mol_type = other DNA
atgaaaatggaagagctgttcaaaaaacacaaaatcgttgcggtactgcgcgcaaattccgtcgaagaggctaaaaaaaaagctctggctgttttcctgggtggcgtgcatctgatcgaaatcacctttaccgtacctgatgctgatacggtgatcaaggaactgtctttcctgaaggaaatgggcgctatcatcggtgctggcaccgttaccagcgttgaacaggcacgtaaggctgttgaaagcggcgcggagttcatcgtttctccgcatctggatgaagaaatctcccagttcgcgaaagaaaagggtgtcttctatatgccgggcgtgatgactccaactgaactggtcaaagcgatgaaactgggtcacaccatcctgaaactgtttccaggtgaagtggttggtccacagttcgtgaaagccatgaaaggcccgttccctaacgttaaattcgtcccgaccggcggtgtaaacctggataacgtttgcgaatggttcaaagcgggtgtactggctgttggtgttggttccgcactggttaaaggcacgccagtggaagtagctgaaaaagccaaagccttcgtggaaaagatccgtggctgtaccgaa

SEQ ID NO: 31 - DNA, 930 bp, synthetic construct
  source 1..930: mol_type = other DNA
atggactctgctactcacatcaaattctctaaacgcgacgaagacggcaaagaactggcaggcgctactatggaactgcgtgactccagcggcaaaactatctccacttggatctccgacggtcaggtgaaggatttctacctgtacccgggcaaatacaccttcgttgaaactgcagcacctgacggttacgaagtagcaactgctatcacgttcaccgttaacgagcagggtcaggttaccgttaacggcaaggcgactaagggtgatgcacacatcggtggttctggcggctctggtggttctggtggctctatgaaaatggaagagctgttcaaaaaacacaaaatcgttgcggtactgcgcgcaaattccgtcgaagaggctaaaaaaaaagctctggctgttttcctgggtggcgtgcatctgatcgaaatcacctttaccgtacctgatgctgatacggtgatcaaggaactgtctttcctgaaggaaatgggcgctatcatcggtgctggcaccgttaccagcgttgaacaggcacgtaaggctgttgaaagcggcgcggagttcatcgtttctccgcatctggatgaagaaatctcccagttcgcgaaagaaaagggtgtcttctatatgccgggcgtgatgactccaactgaactggtcaaagcgatgaaactgggtcacaccatcctgaaactgtttccaggtgaagtggttggtccacagttcgtgaaagccatgaaaggcccgttccctaacgttaaattcgtcccgaccggcggtgtaaacctggataacgtttgcgaatggttcaaagcgggtgtactggctgttggtgttggttccgcactggttaaaggcacgccagtggaagtagctgaaaaagccaaagccttcgtggaaaagatccgtggctgtaccgaa